European Patent Application EP 4 632 065 A1, published October 15, 2025. Title: Novel CRISPR-Cas δ enzyme and system. Applicant: CHINA AGRICULTURAL UNIVERSITY. Application WO. The sequence listing filed with the application follows.

SEQUENCE LISTING (67 sequences)

SEQ ID NO: 1 - protein, 936 aa, synthetic construct
MSKDGDKMKHSKQEVSEDKGVKKDPSVFRCQNLAILEMREEVADYYADLQADYRHYLPLMILWGQNGFMEPDETGLNFSAVLPSTAKTRCENRYGAQIAADLKLIADDLPSSLYAIFTNDYQPLTGVKKVGDRWKFVTSLNTVSDEEFAKKVKPLLRDYKGVTEEQWRRFREERVAGKTADQVWDDLDSILRNPTLAALKKIHDKHMFRVKRPESKLYCDALAHMLSSSYDSWKKINEARQLELQAMRDEQQGLLANKTTNSLYNLVCEFADELESQNYGLTRRIFFIARKEWEDEKSHYLPVIKLLVTEKYLPLLQADNKTVSPAVKAWDICSTLKQRSPYIRFVPPTKDYPIPFGQTGRGHKFTLKEEAGKVCFLVPGLTKDEMPLSGSHYFSSLRIDKVGTDFKISFRHKTKIRSKKSARVTVKQPRINGTVTEVGILRRNGKFFLRVAYKIAYPQHNIDLKSYFASAAPSTQKLELLPAQMRVAGVDLNISDPIVVSKADIFKGEDGGPLSVLDYGSGKVVGEPVIICKDTSRAGKISSLATKCRTLRDVIRNFRHSLHQGTPLPSKSLEFLQEVPVAQEDLKSPSPRYLIQTWIKYIRTEMKRLHYKVWLDGYCHTSEAMRMLDLVDQVAFLMKSYENIHVKPGHKIPKKTTASLKIRETSRTRFRLHVSRLVGARVVRACEDCQMIFLEDLSTGFSEGSNNSLARLFSAGQLKNSIVMAAEKVGKAVVFVCKDGTSIKDPVFGLHGLRPSKKTPGIPPDKKRLYVRRDGKIGYINADQAASLNVLLVGLSHSVAKYKFFVKDGKLQDDEEVAAQQGKKPRKIGVRLERLLKMNFDTPARLFFSLEKDQVVPCYEATETPYTGWVYVYHDRLLTTRQRDQQVNQLAQEVKDLLRDGVKIPKWDVIPDCDNSCLGFSPCLVLDDETAAVSVV

SEQ ID NO: 2 - protein, 867 aa, synthetic construct
MELKTTFCQSLKIKILPESHKLYYDELQADLKKMRIFFATHSGLNYSYKEDENDSEWKIASSKKSTLSPEAQRLIDIIAKGGIGAEHAYGIFYKDKKVSDKIRRDNSNCIFAMLLPNLVNFEEEYKKRKSKLQLTKEEWEEYHKRCLAGESVEVLWSEEIAPKIGPNEAARLASLAYHQFPDSRHPADITHCRALMSMVADSFCSWVECHKLHREETEKLKTKLQEKIESCKEAYNLLLAYSEDLYSRNYGLSARVLKALIDNKSRCCFDIAFQIAEKYPALMKIDEKTLFKAYNALKLHWKIKRRKPFISLPKIERDYQVPFGLTGSRGKKFDVYVENKNIVVEIDGQKVETFSSHYFSDMQISKIYGEKKNLKGFKLKFRHKLKDKKKEVYGEWIEAELKEIKIKKDMETGDFYLYLPYTTTHNEKNLLLEKFFSYADPLKETIFKNGKTELPNEFLGFGFDLNLSDPIAMAVAEFVRDSSDGEIGALDYGHGKLLDASVLVCNSSLSKRINDLVGDNRKLIQAIRSYKNSLVTKEMDEESGEWLKKALGNAKYGNHRHQLQLVMSKLNKKSKKYWQECRKNGHNDLSENIALLKLLDVQFSLHKSYNNIHIFDYKKQIHSHKTDSKRENFREFVTKQFAATIVKHCKEVMAKYGREYAVVFLEDLEMYFDADADNNSLIRLFAPGQLKKYIASALAKSKIGYVFIPPAGTSKTDPLTSKIGFRATGKYYKQLGYLLNKSDLYVERNGVIGKINSDVAAAINILLKGVNHSIVPYRFLNKHAGSEQKRLKRFEGEIGCDLKKMPKTRLYYLDGKIITEEEKNSLEEALLAEIKHFLLSKANIPEFDAIPGSNGTCKAFSVPRCLK

SEQ ID NO: 3 - protein, 905 aa, synthetic construct
NLAILEMREEVADYYADLQADYRHYLPLMILWGQNGFMEPDETGLNFSAVLPSTAKTRCENRYGAQIAADLKLIADDLPSSLYAIFTNDYQPLTGVKKVGDRWKFVTSLNTVSDEEFAKKVKPLLRDYKGVTEEQWRRFREERVAGKTADQVWDDLDSILRNPTLAALKKIHDKHMFRVKRPESKLYCDALAHMLSSSYDSWKKINEARQLELQAMRDEQQGLLANKTTNSLYNLVCEFADELESQNYGLTRRIFFIARKEWEDEKSHYLPVIKLLVTEKYLPLLQADNKTVSPAVKAWDICSTLKQRSPYIRFVPPTKDYPIPFGQTGRGHKFTLKEEAGKVCFLVPGLTKDEMPLSGSHYFSSLRIDKVGTDFKISFRHKTKIRSKKSARVTVKQPRINGTVTEVGILRRNGKFFLRVAYKIAYPQHNIDLKSYFASAAPSTQKLELLPAQMRVAGVDLNISDPIVVSKADIFKGEDGGPLSVLDYGSGKVVGEPVIICKDTSRAGKISSLATKCRTLRDVIRNFRHSLHQGTPLPSKSLEFLQEVPVAQEDLKSPSPRYLIQTWIKYIRTEMKRLHYKVWLDGYCHTSEAMRMLDLVDQVAFLMKSYENIHVKPGHKIPKKTTASLKIRETSRTRFRLHVSRLVGARVVRACEDCQMIFLEDLSTGFSEGSNNSLARLFSAGQLKNSIVMAAEKVGKAVVFVCKDGTSIKDPVFGLHGLRPSKKTPGIPPDKKRLYVRRDGKIGYINADQAASLNVLLVGLSHSVAKYKFFVKDGKLQDDEEVAAQQGKKPRKIGVRLERLLKMNFDTPARLFFSLEKDQVVPCYEATETPYTGWVYVYHDRLLTTRQRDQQVNQLAQEVKDLLRDGVKIPKWDVIPDCDNSCLGFSPCLVLDDETAAVSVV

SEQ ID NO: 4 - DNA, 2811 bp, synthetic construct
  source 1..2811: mol_type = other DNA
atgtccaaagacggtgacaagatgaagcacagcaaacaagaagtctctgaggacaaaggggtcaagaaagacccgtctgtcttccgctgtcagaacctcgcgattctggagatgcgtgaagaagtcgctgattactacgccgaccttcaggccgactaccgtcactacttgcccctgatgatcctctggggccagaacgggttcatggagccagacgaaactggtctgaacttcagtgccgtcctgccatcgaccgcaaaaacacggtgcgagaaccgctacggtgcgcagattgcggctgatctcaagttgatcgccgacgatctcccgagcagtctctatgccatcttcaccaacgactaccagcccctcaccggcgtgaagaaggtcggcgacagatggaagttcgtcacgtccctcaacactgtcagcgacgaagagttcgccaagaaggtgaagccgctcctgcgtgactacaaaggcgttaccgaagagcagtggcgtcgatttcgtgaagagcgtgtcgccggcaagacagccgatcaggtctgggacgaccttgacagcattctgcgaaacccgacgctcgcggccctgaagaagatccacgacaagcacatgttccgggtcaagcgacccgagagcaaactctactgtgacgccctggctcacatgctgagttccagctacgacagttggaagaaaatcaacgaggcccgccaactcgaactccaagccatgcgtgacgagcagcagggcttgctcgccaacaagaccacgaacagtctgtacaatctggtgtgcgagttcgccgacgaactggagtcgcagaactacggtctgactcggcggatcttcttcatcgcccgcaaagagtgggaggacgaaaagtcccattacctcccggtcatcaagctcctcgtcacggagaagtatctgcccctgctccaggcggataacaagactgtcagccccgccgtcaaggcgtgggacatctgctctactctgaagcagaggtcgccgtacatccgcttcgtgcctccgaccaaggactatccgatccccttcggccagacgggtcgcggacacaagttcaccttgaaagaggaagccggaaaggtctgtttcctcgtacccggcctgaccaaggacgagatgcctctgtccggctctcactacttctcaagcctccgtatcgacaaggtcggcacagacttcaagatctcgttccgtcacaagaccaagattcgcagcaaaaagtctgcgcgagtcaccgtcaagcagcccaggatcaacggcaccgtcactgaggtcggcatcctacgcaggaacggcaagttcttcctgcgtgtcgcttacaagatcgcctacccacagcacaacatcgacctgaagagctacttcgcctcggcagccccctccacgcaaaagctggagcttctgccggctcaaatgagagtcgcgggcgtcgatctgaacatcagcgacccgattgtcgtctccaaggccgacatcttcaagggcgaagacggcgggccgctgtctgtgctggactacggctctggcaaggtggtaggtgagcctgtgatcatctgcaaggacaccagcagggccgggaagatcagttccctcgccacgaaatgccggacgctacgcgacgtgatccgcaactttcgtcattcactgcatcagggtacgcccttgcccagcaagagtcttgaatttctccaagaagttcccgtggcgcaggaggacttgaagtcgcccagccctcgctatctgatccagacgtggatcaagtacatcaggaccgagatgaagcgacttcactacaaggtctggctcgacgggtactgccacactagcgaagccatgcggatgctcgatctggtcgatcaggtcgcgttcctaatgaagtcgtatgagaacatccacgtcaaaccgggtcacaagatcccgaagaagaccactgcgtccctgaagattcgcgagacgagccgaacgcggttcaggctgcatgtctcccgacttgtcggtgcgcgagtggttcgtgcgtgcgaggactgccagatgatcttcttggaagatctctcgacaggtttctccgaaggcagcaataactcgttggcccggctgttttcggctggccaactgaagaactccatcgtcatggcggcagagaaggtcggcaaagccgtagtcttcgtgtgcaaggacggtacgtctatcaaagatcctgttttcggtctgcacggcctgcggccttccaagaagaccccaggcattccgccggacaagaagcgtctctacgtccgtcgcgacggcaaaatcggctacatcaacgccgatcaggcggcttcgctgaatgtgctgctggtggggctgtcgcactccgtcgccaagtacaagttctttgtcaaggacgggaagctacaagacgacgaggaggtggctgcccagcaaggcaagaagccgcgtaagatcggtgttcgtctggaaagactcctcaagatgaacttcgacacccctgccagacttttcttctcgctggagaaagatcaggtggtgccgtgctacgaggccacggaaacgccttacaccggctgggtctacgtctaccacgaccgactgctgaccacccggcaacgtgatcagcaagtcaatcaactcgcacaggaagtcaaggatctcctgcgggatggtgtcaaaattcctaaatgggacgtaatcccagactgcgacaacagttgcctcggcttctctccgtgtctggtgcttgacgacgaaaccgccgctgtttctgtggtttag

SEQ ID NO: 5 - DNA, 2604 bp, synthetic construct
  source 1..2604: mol_type = other DNA
atggaattgaagacaactttttgtcagtcactaaaaattaagatcctccccgaaagccataagttgtattacgatgagctgcaagccgacctaaagaagatgagaatcttcttcgcaacgcactctgggctcaactacagctacaaggaagatgaaaacgattcggaatggaagatagcgtcgtcaaaaaagagcacactctcacctgaagcccaaaggcttattgacatcatcgccaaaggcggtataggagcagagcacgcctacggaatattttacaaggacaaaaaggtgtcggacaagatccggcgagataattcaaactgcatcttcgccatgctattacctaacctcgtcaatttcgaggaagaatacaaaaagaggaaaagtaagctccagctcaccaaggaagagtgggaggagtaccataaacgatgtcttgcaggcgagagcgtggaagtcctgtggtccgaggagattgctccaaaaattgggcctaacgaagcggcgagactggcatcactcgcgtatcaccagttcccagattctcgtcatccggcggacattacccactgcagggcgctcatgtctatggtagcagactctttttgttcctgggtcgagtgccacaagctgcaccgtgaggaaacagagaaactcaagacgaaattacaggagaagatagagagctgcaaggaggcatacaatctgctactcgcttattccgaagacctgtacagtaggaattatggtctgagtgccagggttttgaaggcacttattgacaacaaatcccggtgctgcttcgacatagcctttcagatcgcggagaaatatcctgcactgatgaagattgatgaaaagaccctgttcaaggcctacaacgccctaaagctccactggaaaataaaacgacgcaagccgttcatctcgctgcccaagatcgagagggactaccaggtgccctttggactcacaggaagcagaggcaagaagttcgacgtctatgtggaaaacaagaatattgtggtcgagatcgacggccagaaagtcgaaaccttcagctctcactatttctctgatatgcagatctccaagatttacggtgaaaagaaaaatttgaagggattcaagttgaaattccgccacaagctgaaggacaagaagaaggaggtttatggagagtggattgaggcggagctgaaggaaatcaagattaagaaagacatggagacaggcgacttctacctgtatctcccatacactacaacgcataatgagaaaaacttattgctcgagaagttcttttcctacgccgatccacttaaggagactatttttaagaacggaaagacggagcttccaaatgaatttctaggcttcggcttcgatttgaacctttccgacccgattgcgatggcggttgccgagtttgttcgggactcatcagatggtgagattggcgccctcgactatggtcacggtaagctcctcgacgctagtgttttggtctgcaactcatcactatcaaagcgcatcaatgacctggttggagacaatagaaagctgatccaagctattagatcgtacaagaactcgctagtaactaaggaaatggacgaggagagtggcgagtggcttaaaaaagctctaggcaatgcaaagtacggcaaccataggcatcagcttcaactggtcatgtctaagctgaacaaaaaaagcaaaaagtactggcaggaatgtcgcaagaacggccacaacgatctttccgaaaatattgcactattaaagttgttggacgtgcagttctctttgcataaaagctataacaacatacacatctttgattacaaaaaacaaattcacagccataagactgactccaaaagggagaatttccgtgaatttgtgacgaagcaatttgcggctaccatagtaaagcattgcaaggaggtgatggctaaatatggcagagagtacgccgttgtctttttggaggacctggagatgtactttgatgctgatgctgataacaattctctgatccggctttttgcacccggccaattgaagaagtacatcgcctccgctctggctaagagcaagataggttatgtgttcatccctcctgctgggacaagtaagaccgacccgttaacttcgaaaattggattcagggctaccggaaaatactacaagcagctgggctatctgcttaataagtccgacctctacgtggagcgcaacggggttatcgggaagatcaacagtgatgtagctgcggcgataaatattctcttaaagggcgtgaaccactcaatcgtgccgtaccgcttcctgaataaacatgctgggtctgaacagaagcgcctcaaacgttttgaaggggagatcggttgtgatctgaaaaagatgccaaagacacgcctctactatcttgacggaaaaatcatcactgaagaggagaagaacagcctggaggaagcgctactcgctgagatcaagcacttccttctgtcgaaggccaacattccggagtttgatgcaataccggggagcaatggcacctgcaaagccttctccgttccacgctgccttaagtga

SEQ ID NO: 6 - DNA, 2718 bp, synthetic construct
  source 1..2718: mol_type = other DNA
aacctcgcgattctggagatgcgtgaagaagtcgctgattactacgccgaccttcaggccgactaccgtcactacttgcccctgatgatcctctggggccagaacgggttcatggagccagacgaaactggtctgaacttcagtgccgtcctgccatcgaccgcaaaaacacggtgcgagaaccgctacggtgcgcagattgcggctgatctcaagttgatcgccgacgatctcccgagcagtctctatgccatcttcaccaacgactaccagcccctcaccggcgtgaagaaggtcggcgacagatggaagttcgtcacgtccctcaacactgtcagcgacgaagagttcgccaagaaggtgaagccgctcctgcgtgactacaaaggcgttaccgaagagcagtggcgtcgatttcgtgaagagcgtgtcgccggcaagacagccgatcaggtctgggacgaccttgacagcattctgcgaaacccgacgctcgcggccctgaagaagatccacgacaagcacatgttccgggtcaagcgacccgagagcaaactctactgtgacgccctggctcacatgctgagttccagctacgacagttggaagaaaatcaacgaggcccgccaactcgaactccaagccatgcgtgacgagcagcagggcttgctcgccaacaagaccacgaacagtctgtacaatctggtgtgcgagttcgccgacgaactggagtcgcagaactacggtctgactcggcggatcttcttcatcgcccgcaaagagtgggaggacgaaaagtcccattacctcccggtcatcaagctcctcgtcacggagaagtatctgcccctgctccaggcggataacaagactgtcagccccgccgtcaaggcgtgggacatctgctctactctgaagcagaggtcgccgtacatccgcttcgtgcctccgaccaaggactatccgatccccttcggccagacgggtcgcggacacaagttcaccttgaaagaggaagccggaaaggtctgtttcctcgtacccggcctgaccaaggacgagatgcctctgtccggctctcactacttctcaagcctccgtatcgacaaggtcggcacagacttcaagatctcgttccgtcacaagaccaagattcgcagcaaaaagtctgcgcgagtcaccgtcaagcagcccaggatcaacggcaccgtcactgaggtcggcatcctacgcaggaacggcaagttcttcctgcgtgtcgcttacaagatcgcctacccacagcacaacatcgacctgaagagctacttcgcctcggcagccccctccacgcaaaagctggagcttctgccggctcaaatgagagtcgcgggcgtcgatctgaacatcagcgacccgattgtcgtctccaaggccgacatcttcaagggcgaagacggcgggccgctgtctgtgctggactacggctctggcaaggtggtaggtgagcctgtgatcatctgcaaggacaccagcagggccgggaagatcagttccctcgccacgaaatgccggacgctacgcgacgtgatccgcaactttcgtcattcactgcatcagggtacgcccttgcccagcaagagtcttgaatttctccaagaagttcccgtggcgcaggaggacttgaagtcgcccagccctcgctatctgatccagacgtggatcaagtacatcaggaccgagatgaagcgacttcactacaaggtctggctcgacgggtactgccacactagcgaagccatgcggatgctcgatctggtcgatcaggtcgcgttcctaatgaagtcgtatgagaacatccacgtcaaaccgggtcacaagatcccgaagaagaccactgcgtccctgaagattcgcgagacgagccgaacgcggttcaggctgcatgtctcccgacttgtcggtgcgcgagtggttcgtgcgtgcgaggactgccagatgatcttcttggaagatctctcgacaggtttctccgaaggcagcaataactcgttggcccggctgttttcggctggccaactgaagaactccatcgtcatggcggcagagaaggtcggcaaagccgtagtcttcgtgtgcaaggacggtacgtctatcaaagatcctgttttcggtctgcacggcctgcggccttccaagaagaccccaggcattccgccggacaagaagcgtctctacgtccgtcgcgacggcaaaatcggctacatcaacgccgatcaggcggcttcgctgaatgtgctgctggtggggctgtcgcactccgtcgccaagtacaagttctttgtcaaggacgggaagctacaagacgacgaggaggtggctgcccagcaaggcaagaagccgcgtaagatcggtgttcgtctggaaagactcctcaagatgaacttcgacacccctgccagacttttcttctcgctggagaaagatcaggtggtgccgtgctacgaggccacggaaacgccttacaccggctgggtctacgtctaccacgaccgactgctgaccacccggcaacgtgatcagcaagtcaatcaactcgcacaggaagtcaaggatctcctgcgggatggtgtcaaaattcctaaatgggacgtaatcccagactgcgacaacagttgcctcggcttctctccgtgtctggtgcttgacgacgaaaccgccgctgtttctgtggtttag

SEQ ID NO: 7 - RNA, 36 nt, synthetic construct
  source 1..36: mol_type = other RNA
gtgctgacgaccagcactagatggtcgttcaggcac

SEQ ID NO: 8 - RNA, 36 nt, synthetic construct
  source 1..36: mol_type = other RNA
gtgctgaacagggtcgctaggcgttgttcaaggcac

SEQ ID NO: 9 - RNA, 34 nt, synthetic construct
  source 1..34: mol_type = other RNA
gctgacgaccagcactagatggtcgttcaggcac

SEQ ID NO: 10 - RNA, 32 nt, synthetic construct
  source 1..32: mol_type = other RNA
tgacgaccagcactagatggtcgttcaggcac

SEQ ID NO: 11 - RNA, 30 nt, synthetic construct
  source 1..30: mol_type = other RNA
acgaccagcactagatggtcgttcaggcac

SEQ ID NO: 12 - RNA, 28 nt, synthetic construct
  source 1..28: mol_type = other RNA
gaccagcactagatggtcgttcaggcac

SEQ ID NO: 13 - RNA, 26 nt, synthetic construct
  source 1..26: mol_type = other RNA
ccagcactagatggtcgttcaggcac

SEQ ID NO: 14 - RNA, 24 nt, synthetic construct
  source 1..24: mol_type = other RNA
agcactagatggtcgttcaggcac

SEQ ID NO: 15 - RNA, 22 nt, synthetic construct
  source 1..22: mol_type = other RNA
cactagatggtcgttcaggcac

SEQ ID NO: 16 - RNA, 20 nt, synthetic construct
  source 1..20: mol_type = other RNA
ctagatggtcgttcaggcac

SEQ ID NO: 17 - DNA, 36 bp, synthetic construct
  source 1..36: mol_type = other DNA
gtgctgacgaccagcactagatggtcgttcaggcac

SEQ ID NO: 18 - DNA, 37 bp, synthetic construct
  source 1..37: mol_type = other DNA
gtgctgaacagggtcgctaggcgttgttcaaggcacg

SEQ ID NO: 19 - DNA, 34 bp, synthetic construct
  source 1..34: mol_type = other DNA
gctgacgaccagcactagatggtcgttcaggcac

SEQ ID NO: 20 - DNA, 32 bp, synthetic construct
  source 1..32: mol_type = other DNA
tgacgaccagcactagatggtcgttcaggcac

SEQ ID NO: 21 - DNA, 30 bp, synthetic construct
  source 1..30: mol_type = other DNA
acgaccagcactagatggtcgttcaggcac

SEQ ID NO: 22 - DNA, 28 bp, synthetic construct
  source 1..28: mol_type = other DNA
gaccagcactagatggtcgttcaggcac

SEQ ID NO: 23 - protein, 26 aa, synthetic construct
CCAGCACTAGATGGTCGTTCAGGCAC

SEQ ID NO: 24 - DNA, 24 bp, synthetic construct
  source 1..24: mol_type = other DNA
agcactagatggtcgttcaggcac

SEQ ID NO: 25 - DNA, 22 bp, synthetic construct
  source 1..22: mol_type = other DNA
cactagatggtcgttcaggcac

SEQ ID NO: 26 - DNA, 20 bp, synthetic construct
  source 1..20: mol_type = other DNA
ctagatggtcgttcaggcac

SEQ ID NO: 27 - protein, 11 aa, synthetic construct
SRADPKKKRKV

SEQ ID NO: 28 - protein, 979 aa, synthetic construct
MGPKKKRKVMDYKDHDGDYKDHDIDYKDDDDKMSKDGDKMKHSKQEVSEDKGVKKDPSVFRCQNLAILEMREEVADYYADLQADYRHYLPLMILWGQNGFMEPDETGLNFSAVLPSTAKTRCENRYGAQIAADLKLIADDLPSSLYAIFTNDYQPLTGVKKVGDRWKFVTSLNTVSDEEFAKKVKPLLRDYKGVTEEQWRRFREERVAGKTADQVWDDLDSILRNPTLAALKKIHDKHMFRVKRPESKLYCDALAHMLSSSYDSWKKINEARQLELQAMRDEQQGLLANKTTNSLYNLVCEFADELESQNYGLTRRIFFIARKEWEDEKSHYLPVIKLLVTEKYLPLLQADNKTVSPAVKAWDICSTLKQRSPYIRFVPPTKDYPIPFGQTGRGHKFTLKEEAGKVCFLVPGLTKDEMPLSGSHYFSSLRIDKVGTDFKISFRHKTKIRSKKSARVTVKQPRINGTVTEVGILRRNGKFFLRVAYKIAYPQHNIDLKSYFASAAPSTQKLELLPAQMRVAGVDLNISDPIVVSKADIFKGEDGGPLSVLDYGSGKVVGEPVIICKDTSRAGKISSLATKCRTLRDVIRNFRHSLHQGTPLPSKSLEFLQEVPVAQEDLKSPSPRYLIQTWIKYIRTEMKRLHYKVWLDGYCHTSEAMRMLDLVDQVAFLMKSYENIHVKPGHKIPKKTTASLKIRETSRTRFRLHVSRLVGARVVRACEDCQMIFLEDLSTGFSEGSNNSLARLFSAGQLKNSIVMAAEKVGKAVVFVCKDGTSIKDPVFGLHGLRPSKKTPGIPPDKKRLYVRRDGKIGYINADQAASLNVLLVGLSHSVAKYKFFVKDGKLQDDEEVAAQQGKKPRKIGVRLERLLKMNFDTPARLFFSLEKDQVVPCYEATETPYTGWVYVYHDRLLTTRQRDQQVNQLAQEVKDLLRDGVKIPKWDVIPDCDNSCLGFSPCLVLDDETAAVSVVSRADPKKKRKV

SEQ ID NO: 29 - protein, 910 aa, synthetic construct
MGPKKKRKVMDYKDHDGDYKDHDIDYKDDDDKMELKTTFCQSLKIKILPESHKLYYDELQADLKKMRIFFATHSGLNYSYKEDENDSEWKIASSKKSTLSPEAQRLIDIIAKGGIGAEHAYGIFYKDKKVSDKIRRDNSNCIFAMLLPNLVNFEEEYKKRKSKLQLTKEEWEEYHKRCLAGESVEVLWSEEIAPKIGPNEAARLASLAYHQFPDSRHPADITHCRALMSMVADSFCSWVECHKLHREETEKLKTKLQEKIESCKEAYNLLLAYSEDLYSRNYGLSARVLKALIDNKSRCCFDIAFQIAEKYPALMKIDEKTLFKAYNALKLHWKIKRRKPFISLPKIERDYQVPFGLTGSRGKKFDVYVENKNIVVEIDGQKVETFSSHYFSDMQISKIYGEKKNLKGFKLKFRHKLKDKKKEVYGEWIEAELKEIKIKKDMETGDFYLYLPYTTTHNEKNLLLEKFFSYADPLKETIFKNGKTELPNEFLGFGFDLNLSDPIAMAVAEFVRDSSDGEIGALDYGHGKLLDASVLVCNSSLSKRINDLVGDNRKLIQAIRSYKNSLVTKEMDEESGEWLKKALGNAKYGNHRHQLQLVMSKLNKKSKKYWQECRKNGHNDLSENIALLKLLDVQFSLHKSYNNIHIFDYKKQIHSHKTDSKRENFREFVTKQFAATIVKHCKEVMAKYGREYAVVFLEDLEMYFDADADNNSLIRLFAPGQLKKYIASALAKSKIGYVFIPPAGTSKTDPLTSKIGFRATGKYYKQLGYLLNKSDLYVERNGVIGKINSDVAAAINILLKGVNHSIVPYRFLNKHAGSEQKRLKRFEGEIGCDLKKMPKTRLYYLDGKIITEEEKNSLEEALLAEIKHFLLSKANIPEFDAIPGSNGTCKAFSVPRCLKSRADPKKKRKV

SEQ ID NO: 30 - protein, 948 aa, synthetic construct
MGPKKKRKVMDYKDHDGDYKDHDIDYKDDDDKNLAILEMREEVADYYADLQADYRHYLPLMILWGQNGFMEPDETGLNFSAVLPSTAKTRCENRYGAQIAADLKLIADDLPSSLYAIFTNDYQPLTGVKKVGDRWKFVTSLNTVSDEEFAKKVKPLLRDYKGVTEEQWRRFREERVAGKTADQVWDDLDSILRNPTLAALKKIHDKHMFRVKRPESKLYCDALAHMLSSSYDSWKKINEARQLELQAMRDEQQGLLANKTTNSLYNLVCEFADELESQNYGLTRRIFFIARKEWEDEKSHYLPVIKLLVTEKYLPLLQADNKTVSPAVKAWDICSTLKQRSPYIRFVPPTKDYPIPFGQTGRGHKFTLKEEAGKVCFLVPGLTKDEMPLSGSHYFSSLRIDKVGTDFKISFRHKTKIRSKKSARVTVKQPRINGTVTEVGILRRNGKFFLRVAYKIAYPQHNIDLKSYFASAAPSTQKLELLPAQMRVAGVDLNISDPIVVSKADIFKGEDGGPLSVLDYGSGKVVGEPVIICKDTSRAGKISSLATKCRTLRDVIRNFRHSLHQGTPLPSKSLEFLQEVPVAQEDLKSPSPRYLIQTWIKYIRTEMKRLHYKVWLDGYCHTSEAMRMLDLVDQVAFLMKSYENIHVKPGHKIPKKTTASLKIRETSRTRFRLHVSRLVGARVVRACEDCQMIFLEDLSTGFSEGSNNSLARLFSAGQLKNSIVMAAEKVGKAVVFVCKDGTSIKDPVFGLHGLRPSKKTPGIPPDKKRLYVRRDGKIGYINADQAASLNVLLVGLSHSVAKYKFFVKDGKLQDDEEVAAQQGKKPRKIGVRLERLLKMNFDTPARLFFSLEKDQVVPCYEATETPYTGWVYVYHDRLLTTRQRDQQVNQLAQEVKDLLRDGVKIPKWDVIPDCDNSCLGFSPCLVLDDETAAVSVVSRADPKKKRKV

SEQ ID NO: 31 - DNA, 2967 bp, synthetic construct
  source 1..2967: mol_type = other DNA
atgggaccaaagaagaagagaaaggttatggattacaaggaccacgacggagactataaagatcatgacatcgattataaggatgatgatgacaagatgtctaaagacggggacaaaatgaaacactccaagcaagaagtttccgaggacaaaggcgtcaagaaagatccgtccgtgtttcgatgccagaacctcgccatactcgagatgagggaggaggtcgctgactattacgcagaccttcaggctgactaccggcactacctgcctctgatgattctgtgggggcaaaatggctttatggagccagatgaaacgggcctcaacttcagcgccgtcctgccgtcgaccgcgaaaacacgctgtgagaataggtatggtgcccagattgcagccgacctgaaactcatcgcagatgatctgccgtctagcctgtatgctatattcacgaatgattaccagcctttaactggcgtgaagaaggttggtgaccgttggaagtttgtgacttcattgaacaccgtgtcggatgaggaatttgcaaagaaagtcaaacccctccttcgcgactacaaaggtgtcacagaggagcagtggcgtcgtttccgtgaggaacgagttgctgggaaaacagccgaccaggtttgggacgatctcgattccatcttgaggaacccgacgcttgccgccctcaaaaagattcatgacaagcacatgttcagagttaagaggccggagtcaaagctgtattgtgatgcattggcgcatatgctctcatcttcatatgattcatggaaaaagatcaatgaagcacgtcagttggaactacaggccatgagagacgaacaacaaggcctgctggcaaataaaactactaactctctttacaatctggtctgtgagttcgcggatgagcttgaatcacaaaactacggcctgacccgaaggatattcttcatcgccaggaaagagtgggaggatgaaaagtcgcactaccttcctgtgatcaaactcttggtgaccgagaagtatcttccacttctgcaggcggataacaaaacagtttctccggcggttaaggcgtgggatatttgcagcacgttgaagcagcgcagtccatatatacggttcgttcctcccacaaaagactatccgattccatttggccagacaggtaggggacacaagtttacactcaaggaggaggccgggaaggtttgcttcctggttccaggactcaccaaggatgaaatgccactctcgggctcccactatttctctagtctgcgaattgacaaggtcggcacagacttcaagatcagcttccgccataagacgaagattcgaagcaagaagtcagctagagtgaccgtaaaacaacctcggatcaacggcaccgttacggaggtgggtatcctgcgtcgcaacggcaagtttttcttacgggttgcgtacaagattgcttacccgcaacacaacattgatcttaagagctacttcgccagcgccgccccttccactcagaagctcgagctgctccctgctcagatgagggtggcgggagtcgatttgaacatttccgatcccatcgtcgtatccaaagctgatatttttaagggagaggatggagggccattatcggtcttggactacggatctggcaaggtagtgggcgagcccgtcatcatctgtaaggatacaagtcgcgcaggtaaaatctcctcgctcgcgactaagtgccgcaccttaagagacgtcattcggaatttccgccactctctccatcagggaacccccctacccagtaagagcctggagtttctgcaggaggtgccagtggcccaggaggacctaaaatcgccatcccccaggtatctcatacagacctggataaagtatatcagaacagagatgaagcgcttgcattataaagtgtggttggacggctactgccacacatctgaagctatgcgtatgcttgatctagttgatcaggtcgccttcctcatgaagtcatacgaaaacatacatgtgaagccgggccataaaattcccaagaaaactaccgcgagtctcaagattagggaaacatccaggacgagatttagactgcatgtatccaggttggtcggggccagggtggtccgcgcctgtgaagattgtcagatgatcttcctggaagacttgtcgaccggcttctcagaaggtagcaacaatagcctcgcgcggctgtttagcgccggccagctgaagaatagtatagtgatggcggcggagaaggtgggtaaagctgttgtatttgtctgcaaggatggaactagcataaaggaccctgtcttcggtttacacggccttcggccgtcgaaaaagaccccaggcatccctccggataaaaaaagactttatgtgagacgggatggtaagattgggtacatcaatgctgatcaagctgcaagtctgaatgtactattggtaggtctgagccatagtgtggccaagtacaagttcttcgtcaaagatggtaagttgcaggatgacgaagaggtggcggcacaacaaggaaagaagcctaggaagattggcgttcgcctggaaagactactaaagatgaattttgataccccggcccgccttttttttagcctggagaaggaccaggtggttccgtgctacgaggcgactgagacgccttacacgggttgggtgtacgtctaccatgacaggcttctcacaacacgccagagggaccaacaggtgaatcaacttgcccaagaggtgaaagacttacttagggacggggtgaagatccctaaatgggacgtgatcccagactgcgacaacagttgcctcgggttctctccctgcctggtgcttgacgacgagactgctgctgtctcagttgttggatctgggagcaagcggcccgcagcaacgaaaaaggcagggcaagcaaaaaagaagaaatga

SEQ ID NO: 32 - DNA, 2760 bp, synthetic construct
  source 1..2760: mol_type = other DNA
atgggtccgaaaaagaagcggaaagttatggattataaggatcatgatggcgactataaggatcatgacatagattataaagatgatgacgacaaaatggaattgaagacaactttttgtcagtcactaaaaattaagatcctccccgaaagccataagttgtattacgatgagctgcaagccgacctaaagaagatgagaatcttcttcgcaacgcactctgggctcaactacagctacaaggaagatgaaaacgattcggaatggaagatagcgtcgtcaaaaaagagcacactctcacctgaagcccaaaggcttattgacatcatcgccaaaggcggtataggagcagagcacgcctacggaatattttacaaggacaaaaaggtgtcggacaagatccggcgagataattcaaactgcatcttcgccatgctattacctaacctcgtcaatttcgaggaagaatacaaaaagaggaaaagtaagctccagctcaccaaggaagagtgggaggagtaccataaacgatgtcttgcaggcgagagcgtggaagtcctgtggtccgaggagattgctccaaaaattgggcctaacgaagcggcgagactggcatcactcgcgtatcaccagttcccagattctcgtcatccggcggacattacccactgcagggcgctcatgtctatggtagcagactctttttgttcctgggtcgagtgccacaagctgcaccgtgaggaaacagagaaactcaagacgaaattacaggagaagatagagagctgcaaggaggcatacaatctgctactcgcttattccgaagacctgtacagtaggaattatggtctgagtgccagggttttgaaggcacttattgacaacaaatcccggtgctgcttcgacatagcctttcagatcgcggagaaatatcctgcactgatgaagattgatgaaaagaccctgttcaaggcctacaacgccctaaagctccactggaaaataaaacgacgcaagccgttcatctcgctgcccaagatcgagagggactaccaggtgccctttggactcacaggaagcagaggcaagaagttcgacgtctatgtggaaaacaagaatattgtggtcgagatcgacggccagaaagtcgaaaccttcagctctcactatttctctgatatgcagatctccaagatttacggtgaaaagaaaaatttgaagggattcaagttgaaattccgccacaagctgaaggacaagaagaaggaggtttatggagagtggattgaggcggagctgaaggaaatcaagattaagaaagacatggagacaggcgacttctacctgtatctcccatacactacaacgcataatgagaaaaacttattgctcgagaagttcttttcctacgccgatccacttaaggagactatttttaagaacggaaagacggagcttccaaatgaatttctaggcttcggcttcgatttgaacctttccgacccgattgcgatggcggttgccgagtttgttcgggactcatcagatggtgagattggcgccctcgactatggtcacggtaagctcctcgacgctagtgttttggtctgcaactcatcactatcaaagcgcatcaatgacctggttggagacaatagaaagctgatccaagctattagatcgtacaagaactcgctagtaactaaggaaatggacgaggagagtggcgagtggcttaaaaaagctctaggcaatgcaaagtacggcaaccataggcatcagcttcaactggtcatgtctaagctgaacaaaaaaagcaaaaagtactggcaggaatgtcgcaagaacggccacaacgatctttccgaaaatattgcactattaaagttgttggacgtgcagttctctttgcataaaagctataacaacatacacatctttgattacaaaaaacaaattcacagccataagactgactccaaaagggagaatttccgtgaatttgtgacgaagcaatttgcggctaccatagtaaagcattgcaaggaggtgatggctaaatatggcagagagtacgccgttgtctttttggaggacctggagatgtactttgatgctgatgctgataacaattctctgatccggctttttgcacccggccaattgaagaagtacatcgcctccgctctggctaagagcaagataggttatgtgttcatccctcctgctgggacaagtaagaccgacccgttaacttcgaaaattggattcagggctaccggaaaatactacaagcagctgggctatctgcttaataagtccgacctctacgtggagcgcaacggggttatcgggaagatcaacagtgatgtagctgcggcgataaatattctcttaaagggcgtgaaccactcaatcgtgccgtaccgcttcctgaataaacatgctgggtctgaacagaagcgcctcaaacgttttgaaggggagatcggttgtgatctgaaaaagatgccaaagacacgcctctactatcttgacggaaaaatcatcactgaagaggagaagaacagcctggaggaagcgctactcgctgagatcaagcacttccttctgtcgaaggccaacattccggagtttgatgcaataccggggagcaatggcacctgcaaagccttctccgttccacgctgccttaagggcagcgggagcaagcggcccgccgcgaccaaaaaagcggggcaagccaagaagaaaaagtga

SEQ ID NO: 33 - DNA, 2874 bp, synthetic construct
  source 1..2874: mol_type = other DNA
atgggaccaaagaagaagagaaaggttatggattacaaggaccacgacggagactataaagatcatgacatcgattataaggatgatgatgacaagaacctcgccatactcgagatgagggaggaggtcgctgactattacgcagaccttcaggctgactaccggcactacctgcctctgatgattctgtgggggcaaaatggctttatggagccagatgaaacgggcctcaacttcagcgccgtcctgccgtcgaccgcgaaaacacgctgtgagaataggtatggtgcccagattgcagccgacctgaaactcatcgcagatgatctgccgtctagcctgtatgctatattcacgaatgattaccagcctttaactggcgtgaagaaggttggtgaccgttggaagtttgtgacttcattgaacaccgtgtcggatgaggaatttgcaaagaaagtcaaacccctccttcgcgactacaaaggtgtcacagaggagcagtggcgtcgtttccgtgaggaacgagttgctgggaaaacagccgaccaggtttgggacgatctcgattccatcttgaggaacccgacgcttgccgccctcaaaaagattcatgacaagcacatgttcagagttaagaggccggagtcaaagctgtattgtgatgcattggcgcatatgctctcatcttcatatgattcatggaaaaagatcaatgaagcacgtcagttggaactacaggccatgagagacgaacaacaaggcctgctggcaaataaaactactaactctctttacaatctggtctgtgagttcgcggatgagcttgaatcacaaaactacggcctgacccgaaggatattcttcatcgccaggaaagagtgggaggatgaaaagtcgcactaccttcctgtgatcaaactcttggtgaccgagaagtatcttccacttctgcaggcggataacaaaacagtttctccggcggttaaggcgtgggatatttgcagcacgttgaagcagcgcagtccatatatacggttcgttcctcccacaaaagactatccgattccatttggccagacaggtaggggacacaagtttacactcaaggaggaggccgggaaggtttgcttcctggttccaggactcaccaaggatgaaatgccactctcgggctcccactatttctctagtctgcgaattgacaaggtcggcacagacttcaagatcagcttccgccataagacgaagattcgaagcaagaagtcagctagagtgaccgtaaaacaacctcggatcaacggcaccgttacggaggtgggtatcctgcgtcgcaacggcaagtttttcttacgggttgcgtacaagattgcttacccgcaacacaacattgatcttaagagctacttcgccagcgccgccccttccactcagaagctcgagctgctccctgctcagatgagggtggcgggagtcgatttgaacatttccgatcccatcgtcgtatccaaagctgatatttttaagggagaggatggagggccattatcggtcttggactacggatctggcaaggtagtgggcgagcccgtcatcatctgtaaggatacaagtcgcgcaggtaaaatctcctcgctcgcgactaagtgccgcaccttaagagacgtcattcggaatttccgccactctctccatcagggaacccccctacccagtaagagcctggagtttctgcaggaggtgccagtggcccaggaggacctaaaatcgccatcccccaggtatctcatacagacctggataaagtatatcagaacagagatgaagcgcttgcattataaagtgtggttggacggctactgccacacatctgaagctatgcgtatgcttgatctagttgatcaggtcgccttcctcatgaagtcatacgaaaacatacatgtgaagccgggccataaaattcccaagaaaactaccgcgagtctcaagattagggaaacatccaggacgagatttagactgcatgtatccaggttggtcggggccagggtggtccgcgcctgtgaagattgtcagatgatcttcctggaagacttgtcgaccggcttctcagaaggtagcaacaatagcctcgcgcggctgtttagcgccggccagctgaagaatagtatagtgatggcggcggagaaggtgggtaaagctgttgtatttgtctgcaaggatggaactagcataaaggaccctgtcttcggtttacacggccttcggccgtcgaaaaagaccccaggcatccctccggataaaaaaagactttatgtgagacgggatggtaagattgggtacatcaatgctgatcaagctgcaagtctgaatgtactattggtaggtctgagccatagtgtggccaagtacaagttcttcgtcaaagatggtaagttgcaggatgacgaagaggtggcggcacaacaaggaaagaagcctaggaagattggcgttcgcctggaaagactactaaagatgaattttgataccccggcccgccttttttttagcctggagaaggaccaggtggttccgtgctacgaggcgactgagacgccttacacgggttgggtgtacgtctaccatgacaggcttctcacaacacgccagagggaccaacaggtgaatcaacttgcccaagaggtgaaagacttacttagggacggggtgaagatccctaaatgggacgtgatcccagactgcgacaacagttgcctcgggttctctccctgcctggtgcttgacgacgagactgctgctgtctcagttgttggatctgggagcaagcggcccgcagcaacgaaaaaggcagggcaagcaaaaaagaagaaatga

SEQ ID NO: 34 - DNA, 35 bp, synthetic construct
  source 1..35: mol_type = other DNA
nnnnnnnnggtataacaacttcgacgagctctaca

SEQ ID NO: 35 - RNA, 27 nt, synthetic construct
  source 1..27: mol_type = other RNA
ggtataacaacttcgacgagctctaca

SEQ ID NO: 36 - RNA, 27 nt, synthetic construct
  source 1..27: mol_type = other RNA
ggtataacaacttcgacgagctctaca

SEQ ID NO: 37 - RNA, 26 nt, synthetic construct
  source 1..26: mol_type = other RNA
cggtgggctggcgctggggttcagct

SEQ ID NO: 38 - RNA, 26 nt, synthetic construct
  source 1..26: mol_type = other RNA
gagccagagaggatcctgggagggag

SEQ ID NO: 39 - RNA, 26 nt, synthetic construct
  source 1..26: mol_type = other RNA
tgactttgtcacagcccaagatagtt

SEQ ID NO: 40 - RNA, 26 nt, synthetic construct
  source 1..26: mol_type = other RNA
aaacccagacacatagcaattcagga

SEQ ID NO: 41 - RNA, 26 nt, synthetic construct
  source 1..26: mol_type = other RNA
ctgaggggctgctggtttggctggtg

SEQ ID NO: 42 - RNA, 26 nt, synthetic construct
  source 1..26: mol_type = other RNA
gagatgccagcagaagttgggcagaa

SEQ ID NO: 43 - RNA, 26 nt, synthetic construct
  source 1..26: mol_type = other RNA
gggcagagtggagatggtggggacaa

SEQ ID NO: 44 - RNA, 26 nt, synthetic construct
  source 1..26: mol_type = other RNA
actagggtgggcaaccacaaacccac

SEQ ID NO: 45 - RNA, 26 nt, synthetic construct
  source 1..26: mol_type = other RNA
tgtacagaaggctgaaaggagagaac

SEQ ID NO: 46 - RNA, 26 nt, synthetic construct
  source 1..26: mol_type = other RNA
cggtaccagtttagcacgaagctctc

SEQ ID NO: 47 - RNA, 26 nt, synthetic construct
  source 1..26: mol_type = other RNA
ccaccattgtctttcctagcggaatg

SEQ ID NO: 48 - RNA, 26 nt, synthetic construct
  source 1..26: mol_type = other RNA
aagcactgtgggtacgaaggaaatga

SEQ ID NO: 49 - RNA, 26 nt, synthetic construct
  source 1..26: mol_type = other RNA
tgtcacaaagtaaggattctgatgtg

SEQ ID NO: 50 - RNA, 26 nt, synthetic construct
  source 1..26: mol_type = other RNA
ctgttgttgaaggcgtttgcacatgc

SEQ ID NO: 51 - RNA, 26 nt, synthetic construct
  source 1..26: mol_type = other RNA
tctgcaggccagatgagggctccaga

SEQ ID NO: 52 - RNA, 26 nt, synthetic construct
  source 1..26: mol_type = other RNA
gagccagagaggatcctgggagggag

SEQ ID NO: 53 - RNA, 26 nt, synthetic construct
  source 1..26: mol_type = other RNA
gaccactgtgtgggggtaaaggacct

SEQ ID NO: 54 - RNA, 26 nt, synthetic construct
  source 1..26: mol_type = other RNA
cccccatttcctggagccatctctct

SEQ ID NO: 55 - RNA, 26 nt, synthetic construct
  source 1..26: mol_type = other RNA
aaccttagaggttctggcaaggagag

SEQ ID NO: 56 - RNA, 26 nt, synthetic construct
  source 1..26: mol_type = other RNA
agcaaaccttagaggttctggcaagg

SEQ ID NO: 57 - RNA, 26 nt, synthetic construct
  source 1..26: mol_type = other RNA
atggagccagagaggatcctgggagg

SEQ ID NO: 58 - RNA, 26 nt, synthetic construct
  source 1..26: mol_type = other RNA
ggagggaagggggggatgcgtgacct

SEQ ID NO: 59 - RNA, 26 nt, synthetic construct
  source 1..26: mol_type = other RNA
tgacctgcccggttctcagtggccac

SEQ ID NO: 60 - RNA, 26 nt, synthetic construct
  source 1..26: mol_type = other RNA
gagccagagaggatcctgggagggag

SEQ ID NO: 61 - RNA, 24 nt, synthetic construct
  source 1..24: mol_type = other RNA
gagccagagaggatcctgggaggg

SEQ ID NO: 62 - RNA, 22 nt, synthetic construct
  source 1..22: mol_type = other RNA
gagccagagaggatcctgggag

SEQ ID NO: 63 - RNA, 21 nt, synthetic construct
  source 1..21: mol_type = other RNA
gagccagagaggatcctggga

SEQ ID NO: 64 - RNA, 20 nt, synthetic construct
  source 1..20: mol_type = other RNA
gagccagagaggatcctggg

SEQ ID NO: 65 - RNA, 19 nt, synthetic construct
  source 1..19: mol_type = other RNA
gagccagagaggatcctgg

SEQ ID NO: 66 - RNA, 18 nt, synthetic construct
  source 1..18: mol_type = other RNA
gagccagagaggatcctg

SEQ ID NO: 67 - RNA, 16 nt, synthetic construct
  source 1..16: mol_type = other RNA
gagccagagaggatcc